European Patent Application EP 4 140 494 A1, published March 1, 2023. Title: Composition for prevention and treatment of lipid-related metabolic disease comprising lactobacillus plantarum ATG-K2 or lactobacillus plantarum ATG-K6. Applicant: Gachon University of Industry-Academic cooperation Foundation. The sequence listing filed with the application follows.

SEQUENCE LISTING (12 sequences)

SEQ ID NO: 1 - DNA, 19 bp, Artificial Sequence
  Forward primer sequence used for real-time RT-PCR of SREBP-1C
ccctgcgaagtgctcacaa

SEQ ID NO: 2 - DNA, 24 bp, Artificial Sequence
  Reverse primer sequence used for real-time RT-PCR of SREBP-1C
gcgtttctaccacttcaggtttca

SEQ ID NO: 3 - DNA, 23 bp, Artificial Sequence
  Forward primer sequence used for real-time RT-PCR of FAS
gctgctacaaacaggaccatcac

SEQ ID NO: 4 - DNA, 20 bp, Artificial Sequence
  Reverse primer sequence used for real-time RT-PCR of FAS
tcttgctggcctccactgac

SEQ ID NO: 5 - DNA, 20 bp, Artificial Sequence
  Forward primer sequence used for real-time RT-PCR of C/EBPalpha
gccaagaagtcggtggataa

SEQ ID NO: 6 - DNA, 20 bp, Artificial Sequence
  Reverse primer sequence used for real-time RT-PCR of C/EBPalpha
ccttgaccaaggagctctca

SEQ ID NO: 7 - DNA, 20 bp, Artificial Sequence
  Forward primer sequence used for real-time RT-PCR of ACC
caatcctcggcacatggaga

SEQ ID NO: 8 - DNA, 21 bp, Artificial Sequence
  Reverse primer sequence used for real-time RT-PCR of ACC
gctcagccaagcggatgtaga

SEQ ID NO: 9 - DNA, 21 bp, Artificial Sequence
  Forward primer sequence used for real-time RT-PCR of CPT-1
ccatctcttctgcctctatgt

SEQ ID NO: 10 - DNA, 21 bp, Artificial Sequence
  Reverse primer sequence used for real-time RT-PCR of CPT-1
gtcagggtttttctcaaagtc

SEQ ID NO: 11 - DNA, 20 bp, Artificial Sequence
  Forward primer sequence used for real-time RT-PCR of beta-actin
gattactgccctggctccta

SEQ ID NO: 12 - DNA, 20 bp, Artificial Sequence
  Reverse primer sequence used for real-time RT-PCR of beta-actin
tcatcgtactcctgcttgct